European Patent Application EP 4 610 350 A1, published September 3, 2025. Title: Novel variant of phenylalanine:H+ symporter PheP and method for producing L-aromatic amino acid using the same. Applicant: DAESANG CORPORATION. The sequence listing filed with the application follows.

SEQUENCE LISTING (24 sequences)

SEQ ID NO: 1 - DNA, 1377 bp, Escherichia coli
  source 1..1377: mol_type = genomic DNA
gtgaaaaacgcgtcaaccgtatcggaagatactgcgtcgaatcaagagccgacgcttcatcgcggattacataaccgtcatattcaactgattgcgttgggtggcgcaattggtactggtctgtttcttggcattggcccggcgattcagatggcgggtccggctgtattgctgggctacggcgtcgccgggatcatcgctttcctgattatgcgccagcttggcgaaatggtggttgaggagccggtatccggttcatttgcccactttgcctataaatactggggaccgtttgcgggcttcctctctggctggaactactgggtaatgttcgtgctggtgggaatggcagagctgaccgctgcgggcatctatatgcagtactggttcccggatgttccaacgtggatttgggctgccgccttctttattatcatcaacgccgttaacctggtgaacgtgcgcttatatggcgaaaccgagttctggtttgcgttgattaaagtgctggcaatcatcggtatgatcggctttggcctgtggctgctgttttctggtcacggcggcgagaaagccagtatcgacaacctctggcgctacggtggtttcttcgccaccggctggaatgggctgattttgtcgctggcggtaattatgttctccttcggcggtctggagctgattgggattactgccgctgaagcgcgcgatccggaaaaaagcattccaaaagcggtaaatcaggtggtgtatcgcatcctgctgttttacatcggttcactggtggttttactggcgctctatccgtgggtggaagtgaaatccaacagtagcccgtttgtgatgattttccataatctcgacagcaacgtggtagcttctgcgctgaacttcgtcattctggtagcatcgctgtcagtgtataacagcggggtttactctaacagccgcatgctgtttggcctttctgtgcagggtaatgcgccgaagtttttgactcgcgtcagccgtcgcggtgtgccgattaactcgctgatgctttccggagcgatcacttcgctggtggtgttaatcaactatctgctgccgcaaaaagcgtttggtctgctgatggcgctggtggtagcaacgctgctgttgaactggattatgatctgtctggcgcatctgcgttttcgtgcagcgatgcgacgtcaggggcgtgaaacacagtttaaggcgctgctctatccgttcggcaactatctctgcattgccttcctcggcatgattttgctgctgatgtgcacgatggatgatatgcgcttgtcagcgatcctgctgccggtgtggattgtattcctgtttatggcatttaaaacgctgcgtcggaaataa

SEQ ID NO: 2 - protein, 458 aa, Escherichia coli
MKNASTVSEDTASNQEPTLHRGLHNRHIQLIALGGAIGTGLFLGIGPAIQMAGPAVLLGYGVAGIIAFLIMRQLGEMVVEEPVSGSFAHFAYKYWGPFAGFLSGWNYWVMFVLVGMAELTAAGIYMQYWFPDVPTWIWAAAFFIIINAVNLVNVRLYGETEFWFALIKVLAIIGMIGFGLWLLFSGHGGEKASIDNLWRYGGFFATGWNGLILSLAVIMFSFGGLELIGITAAEARDPEKSIPKAVNQVVYRILLFYIGSLVVLLALYPWVEVKSNSSPFVMIFHNLDSNVVASALNFVILVASLSVYNSGVYSNSRMLFGLSVQGNAPKFLTRVSRRGVPINSLMLSGAITSLVVLINYLLPQKAFGLLMALVVATLLLNWIMICLAHLRFRAAMRRQGRETQFKALLYPFGNYLCIAFLGMILLLMCTMDDMRLSAILLPVWIVFLFMAFKTLRRK

SEQ ID NO: 3 - DNA, 1377 bp, synthetic construct
  source 1..1377: mol_type = other DNA
gtgaaaaacgcgtcaaccgtatcggaagatactgcgtcgaatcaagagccgacgcttcatcgcggattacataaccgtcatattcaactgattgcgttgggtggcgcaattggtactggtctgtttcttggcattggcccggcgattcagatggcgggtccggctgtattgctgggctacggcgtcgccgggatcatcgctttcctgattatgcgccagcttggcgaaatggtggttgaggagccggtatccggttcatttgcccactttgcctataaatactggggaccgtttgcgggcttcctctctggctggaactactgggtaatgttcgtgctggtgggaatggcagagctgaccgctgcgggcatctatatgcagtactggttcccggatgttccaacgtggatttgggctgccgccttctttattatcatcaacgccgttaacctggtgaacgtgcgcttatatggcgaaaccgagttctggtttgcgttgattaaagtgctggcaatcatcggtatgatcggctttggcctgtggctgctgttttctggtcacggcggcgagaaagccagtatcgacaacctctggcgctacggtggtttcttcgccaccggctggaatgggctgattttgtcgctggcggtaattatgttctccttcggcggtctggagctgattgggattactgccgctgaagcgcgcgatccggaaaaaagcattccaaaagcggtaaatcaggtggtgtatcgcatcctgctgttttacatcggttcactggtggttttactggcgctctatccgtgggtgaaagtgaaatccaacagtagcccgtttgtgatgattttccataatctcgacagcaacgtggtagcttctgcgctgaacttcgtcattctggtagcatcgctgtcagtgtataacagcggggtttactctaacagccgcatgctgtttggcctttctgtgcagggtaatgcgccgaagtttttgactcgcgtcagccgtcgcggtgtgccgattaactcgctgatgctttccggagcgatcacttcgctggtggtgttaatcaactatctgctgccgcaaaaagcgtttggtctgctgatggcgctggtggtagcaacgctgctgttgaactggattatgatctgtctggcgcatctgcgttttcgtgcagcgatgcgacgtcaggggcgtgaaacacagtttaaggcgctgctctatccgttcggcaactatctctgcattgccttcctcggcatgattttgctgctgatgtgcacgatggatgatatgcgcttgtcagcgatcctgctgccggtgtggattgtattcctgtttatggcatttaaaacgctgcgtcggaaataa

SEQ ID NO: 4 - protein, 458 aa, synthetic construct
VKNASTVSEDTASNQEPTLHRGLHNRHIQLIALGGAIGTGLFLGIGPAIQMAGPAVLLGYGVAGIIAFLIMRQLGEMVVEEPVSGSFAHFAYKYWGPFAGFLSGWNYWVMFVLVGMAELTAAGIYMQYWFPDVPTWIWAAAFFIIINAVNLVNVRLYGETEFWFALIKVLAIIGMIGFGLWLLFSGHGGEKASIDNLWRYGGFFATGWNGLILSLAVIMFSFGGLELIGITAAEARDPEKSIPKAVNQVVYRILLFYIGSLVVLLALYPWVKVKSNSSPFVMIFHNLDSNVVASALNFVILVASLSVYNSGVYSNSRMLFGLSVQGNAPKFLTRVSRRGVPINSLMLSGAITSLVVLINYLLPQKAFGLLMALVVATLLLNWIMICLAHLRFRAAMRRQGRETQFKALLYPFGNYLCIAFLGMILLLMCTMDDMRLSAILLPVWIVFLFMAFKTLRRK

SEQ ID NO: 5 - DNA, 30 bp, synthetic construct
  source 1..30: mol_type = other DNA
caattttattatagtaattgactattatac

SEQ ID NO: 6 - DNA, 40 bp, synthetic construct
  source 1..40: mol_type = other DNA
tgaaatccaacaattttattatagtaattgactattatac

SEQ ID NO: 7 - DNA, 40 bp, synthetic construct
  source 1..40: mol_type = other DNA
ttggatttcactttcacccagttttagagctagaaatagc

SEQ ID NO: 8 - DNA, 30 bp, synthetic construct
  source 1..30: mol_type = other DNA
ctttcacccagttttagagctagaaatagc

SEQ ID NO: 9 - DNA, 21 bp, synthetic construct
  source 1..21: mol_type = other DNA
gagcctgtcggcctacctgct

SEQ ID NO: 10 - DNA, 20 bp, synthetic construct
  source 1..20: mol_type = other DNA
cggccggcatgagcctgtcg

SEQ ID NO: 11 - DNA, 30 bp, synthetic construct
  source 1..30: mol_type = other DNA
atgccggccgcgcttatatggcgaaaccga

SEQ ID NO: 12 - DNA, 25 bp, synthetic construct
  source 1..25: mol_type = other DNA
cgcttatatggcgaaaccgagttct

SEQ ID NO: 13 - DNA, 25 bp, synthetic construct
  source 1..25: mol_type = other DNA
tagagcgccagtaaaaccaccagtg

SEQ ID NO: 14 - DNA, 25 bp, synthetic construct
  source 1..25: mol_type = other DNA
cacccacggatagagcgccagtaaa

SEQ ID NO: 15 - DNA, 30 bp, synthetic construct
  source 1..30: mol_type = other DNA
tccgtgggtggaagtgaaatccaacagtag

SEQ ID NO: 16 - DNA, 25 bp, synthetic construct
  source 1..25: mol_type = other DNA
gaagtgaaatccaacagtagcccgt

SEQ ID NO: 17 - DNA, 25 bp, synthetic construct
  source 1..25: mol_type = other DNA
gatcataatccagttcaacagcagc

SEQ ID NO: 18 - DNA, 25 bp, synthetic construct
  source 1..25: mol_type = other DNA
gcgccagacagatcataatccagtt

SEQ ID NO: 19 - DNA, 33 bp, synthetic construct
  source 1..33: mol_type = other DNA
tgtctggcgcgagctcctgaaaatctcgataac

SEQ ID NO: 20 - DNA, 23 bp, synthetic construct
  source 1..23: mol_type = other DNA
gagctcctgaaaatctcgataac

SEQ ID NO: 21 - DNA, 20 bp, synthetic construct
  source 1..20: mol_type = other DNA
atatgcagtactggttcccg

SEQ ID NO: 22 - DNA, 20 bp, synthetic construct
  source 1..20: mol_type = other DNA
aactgtgtttcacgcccctg

SEQ ID NO: 23 - DNA, 3234 bp, synthetic construct
  source 1..3234: mol_type = other DNA
tttccataggctccgcccccctgacgagcatcacaaaaatcgacgctcaagtcagaggtggcgaaacccgacaggactataaagataccaggcgtttccccctggaagctccctcgtgcgctctcctgttccgaccctgccgcttaccggatacctgtccgcctttctcccttcgggaagcgtggcgctttctcatagctcacgctgtaggtatctcagttcggtgtaggtcgttcgctccaagctgggctgtgtgcacgaaccccccgttcagcccgaccgctgcgccttatccggtaactatcgtcttgagtccaacccggtaagacacgacttatcgccactggcagcagccactggtaacaggattagcagagcgaggtatgtaggcggtgctacagagttcttgaagtggtggcctaactacggctacactagaaggacagtatttggtatctgcgctctgctgaagccagttaccttcggaaaaagagttggtagctcttgatccggcaaacaaaccaccgctggtagcggtggtttttttgtttgcaagcagcagattacgcgcagaaaaaaaggatctcaagaagatcctttgatcttttctacggggtctgacgctcagtggaacgaaaactcacgttaagggattttggtcatgagattatcaaaaaggatcttcacctagatccttttaaattaaaaatgaagttttaaatcaatctaaagtatatatgagtaaacttggtctgacagttaaaagattgacagtataatagtcaattactataataaaattgatgcgcaggtgaaacacctgctgcagttttagagctagaaatagcaagttaaaataaggctagtccgttatcaacttgaaaaagtggcaccgagtcggtgctttttttcgttttccgggacgccctcgcggacgtgctcatagtccacgacgcccgtgattttgtagccctggccgacggccagcaggtaggccgacaggctcatgccggccggagctcctgaaaatctcgataactcaaaaaatacgcccggtagtgatcttatttcattatggtgaaagttggaacctcttaggatcctctagatttaagaaggagatatacataaaactccttctgagctagttctctagcattctattattttgattcgacaccttaataatagcagaaggagtttttacctgtcaaagaaccatcaaacccttgatacacaaggctttgacctaattttgaaaaatgatgttgtttctatatagtatcaagataagaaagaaaaggatttttcgctacgctcaaatcctttcccgtcacgggcttctcagggcgttttatggcgggtctgctatgtggtgctatctgactttttgctgttcagcagttcctgccctctgattttccagtctgaccacttcggattatcccgtgacaggtcattcagactggctaatgcacccagtaaggcagcggtatcatcaacggggtctgacgctcagtggaacgaaaactcacgttaagggattttggtcatgagattatcaaaaaggatcttcacctagatccttttaaattaaaaatgaagttttaaatcaatctaaagtatatatgagtaaacttggtctgacagttaccaatgcttaatcagtgaggcacctatctcagcgatctgtctatttcgttcatccatagttgcctgactccccgtcgtgtagataactacgatacgggagggcttaccatctggccccagtgctgcaatgataccgcgagacccacgctcaccggctccagatttatcagcaataaaccagccagccggaagggccgagcgcagaagtggtcctgcaactttatccgcctccatccagtctattaattgttgccgggaagctagagtaagtagttcgccagttaatagtttgcgcaacgttgttgccattgctacaggcatcgtggtgtcacgctcgtcgtttggtatggcttcattcagctccggttcccaacgatcaaggcgagttacatgatcccccatgttgtgcaaaaaagcggttagctccttcggtcctccgatcgttgtcagaagtaagttggccgcagtgttatcactcatggttatggcagcactgcataattctcttactgtcatgccatccgtaagatgcttttctgtgactggtgagtactcaaccaagtcattctgagaatagtgtatgcggcgaccgagttgctcttgcccggcgtcaatacgggataataccgcgccacatagcagaactttaaaagtgctcatcattggaaaacgttcttcggggcgaaaactctcaaggatcttaccgctgttgagatccagttcgatgtaacccactcgtgcacccaactgatcttcagcatcttttactttcaccagcgtttctgggtgagcaaaaacaggaaggcaaaatgccgcaaaaaagggaataagggcgacacggaaatgttgaatactcatactcttcctttttcaatattattgaagcatttatcagggttattgtctcatgagcggatacatatttgaatgtatttagaaaaataaacaaataggggttccgcgcacatttccccgaaaagtgccaccaaaaaaacacaaaagaccacattttttaatgtggtctttattcttcaactaaagcacccattagttcaacaaacgaaaattggataaagtgggatatttttaaaatatatatttatgttacagtaagctgcctcgcgcgtttcggtgatgacggtgaaaacctctgacacatgcagctcccggagacggtcacagcttgtctgtaagcggatgccgggagcagacaagcccgtcagggcgcgtcagcgggtgttggcgggtgtcggggcgcagccatgacccagtcacgtagcgatagcggagtgtatactggcttaactatgcggcatcagagcagattgtactgagagtgcaccatatgcggtgtgaaataccgcacagatgcgtaaggagaaaataccgcatcaggcgctcttccgcttcctcgctcactgactcgctgcgctcggtcgttcggctgcggcgagcggtatcagctcactcaaaggcggtaatacggttatccacagaatcaggggataacgcaggaaagaacatgtgagcaaaaggccagcaaaaggccaggaaccgtaaaaaggccgcgttgctggcgtt

SEQ ID NO: 24 - DNA, 9656 bp, synthetic construct
  source 1..9656: mol_type = other DNA
aaagccatgacaaaaacgcgtaacaaaagtgtctataatcacggcagaaaagtccacattgattatttgcacggcgtcacactttgctatgccatagcatttttatccataagattagcggatcctacctgacgctttttatcgcaactctctactgtttctccatacccgtttttttgggaattcgagctctaaggaggttataaaaaatggatattaatactgaaactgagatcaagcaaaagcattcactaaccccctttcctgttttcctaatcagcccggcatttcgcgggcgatattttcacagctatttcaggagttcagccatgaacgcttattacattcaggatcgtcttgaggctcagagctgggcgcgtcactaccagcagctcgcccgtgaagagaaagaggcagaactggcagacgacatggaaaaaggcctgccccagcacctgtttgaatcgctatgcatcgatcatttgcaacgccacggggccagcaaaaaatccattacccgtgcgtttgatgacgatgttgagtttcaggagcgcatggcagaacacatccggtacatggttgaaaccattgctcaccaccaggttgatattgattcagaggtataaaacgaatgagtactgcactcgcaacgctggctgggaagctggctgaacgtgtcggcatggattctgtcgacccacaggaactgatcaccactcttcgccagacggcatttaaaggtgatgccagcgatgcgcagttcatcgcattactgatcgttgccaaccagtacggccttaatccgtggacgaaagaaatttacgcctttcctgataagcagaatggcatcgttccggtggtgggcgttgatggctggtcccgcatcatcaatgaaaaccagcagtttgatggcatggactttgagcaggacaatgaatcctgtacatgccggatttaccgcaaggaccgtaatcatccgatctgcgttaccgaatggatggatgaatgccgccgcgaaccattcaaaactcgcgaaggcagagaaatcacggggccgtggcagtcgcatcccaaacggatgttacgtcataaagccatgattcagtgtgcccgtctggccttcggatttgctggtatctatgacaaggatgaagccgagcgcattgtcgaaaatactgcatacactgcagaacgtcagccggaacgcgacatcactccggttaacgatgaaaccatgcaggagattaacactctgctgatcgccctggataaaacatgggatgacgacttattgccgctctgttcccagatatttcgccgcgacattcgtgcatcgtcagaactgacacaggccgaagcagtaaaagctcttggattcctgaaacagaaagccgcagagcagaaggtggcagcatgacaccggacattatcctgcagcgtaccgggatcgatgtgagagctgtcgaacagggggatgatgcgtggcacaaattacggctcggcgtcatcaccgcttcagaagttcacaacgtgatagcaaaaccccgctccggaaagaagtggcctgacatgaaaatgtcctacttccacaccctgcttgctgaggtttgcaccggtgtggctccggaagttaacgctaaagcactggcctggggaaaacagtacgagaacgacgccagaaccctgtttgaattcacttccggcgtgaatgttactgaatccccgatcatctatcgcgacgaaagtatgcgtaccgcctgctctcccgatggtttatgcagtgacggcaacggccttgaactgaaatgcccgtttacctcccgggatttcatgaagttccggctcggtggtttcgaggccataaagtcagcttacatggcccaggtgcagtacagcatgtgggtgacgcgaaaaaatgcctggtactttgccaactatgacccgcgtatgaagcgtgaaggcctgcattatgtcgtgattgagcgggatgaaaagtacatggcgagttttgacgagatcgtgccggagttcatcgaaaaaatggacgaggcactggctgaaattggttttgtatttggggagcaatggcgatgagatctaaagaggagaaaggatctatggataagaaatactcaataggcttagatatcggcacaaatagcgtcggatgggcggtgatcactgatgaatataaggttccgtctaaaaagttcaaggttctgggaaatacagaccgccacagtatcaaaaaaaatcttataggggctcttttatttgacagtggagagacagcggaagcgactcgtctcaaacggacagctcgtagaaggtatacacgtcggaagaatcgtatttgttatctacaggagattttttcaaatgagatggcgaaagtagatgatagtttctttcatcgacttgaagagtcttttttggtggaagaagacaagaagcatgaacgtcatcctatttttggaaatatagtagatgaagttgcttatcatgagaaatatccaactatctatcatctgcgaaaaaaattggtagattctactgataaagcggatttgcgcttaatctatttggccttagcgcatatgattaagtttcgtggtcattttttgattgagggagatttaaatcctgataatagtgatgtggacaaactatttatccagttggtacaaacctacaatcaattatttgaagaaaaccctattaacgcaagtggagtagatgctaaagcgattctttctgcacgattgagtaaatcaagacgattagaaaatctcattgctcagctccccggtgagaagaaaaatggcttatttgggaatctcattgctttgtcattgggtttgacccctaattttaaatcaaattttgatttggcagaagatgctaaattacagctttcaaaagatacttacgatgatgatttagataatttattggcgcaaattggagatcaatatgctgatttgtttttggcagctaagaatttatcagatgctattttactttcagatatcctaagagtaaatactgaaataactaaggctcccctatcagcttcaatgattaaacgctacgatgaacatcatcaagacttgactcttttaaaagctttagttcgacaacaacttccagaaaagtataaagaaatcttttttgatcaatcaaaaaacggatatgcaggttatattgatgggggagctagccaagaagaattttataaatttatcaaaccaattttagaaaaaatggatggtactgaggaattattggtgaaactaaatcgtgaagatttgctgcgcaagcaacggacctttgacaacggctctattccccatcaaattcacttgggtgagctgcatgctattttgagaagacaagaagacttttatccatttttaaaagacaatcgtgagaagattgaaaaaatcttgacttttcgaattccttattatgttggtccattggcgcgtggcaatagtcgttttgcatggatgactcggaagtctgaagaaacaattaccccatggaattttgaagaagttgtcgataaaggtgcttcagctcaatcatttattgaacgcatgacaaactttgataaaaatcttccaaatgaaaaagtactaccaaaacatagtttgctttatgagtattttacggtttataacgaattgacaaaggtcaaatatgttactgaaggaatgcgaaaaccagcatttctttcaggtgaacagaagaaagccattgttgatttactcttcaaaacaaatcgaaaagtaaccgttaagcaattaaaagaagattatttcaaaaaaatagaatgttttgatagtgttgaaatttcaggagttgaagatagatttaatgcttcattaggtacctaccatgatttgctaaaaattattaaagataaagattttttggataatgaagaaaatgaagatatcttagaggatattgttttaacattgaccttatttgaagatagggagatgattgaggaaagacttaaaacatatgctcacctctttgatgataaggtgatgaaacagcttaaacgtcgccgttatactggttggggacgtttgtctcgaaaattgattaatggtattagggataagcaatctggcaaaacaatattagattttttgaaatcagatggttttgccaatcgcaattttatgcagctgatccatgatgatagtttgacatttaaagaagacattcaaaaagcacaagtgtctggacaaggcgatagtttacatgaacatattgcaaatttagctggtagccctgctattaaaaaaggtattttacagactgtaaaagttgttgatgaattggtcaaagtaatggggcggcataagccagaaaatatcgttattgaaatggcacgtgaaaatcagacaactcaaaagggccagaaaaattcgcgagagcgtatgaaacgaatcgaagaaggtatcaaagaattaggaagtcagattcttaaagagcatcctgttgaaaatactcaattgcaaaatgaaaagctctatctctattatctccaaaatggaagagacatgtatgtggaccaagaattagatattaatcgtttaagtgattatgatgtcgatcacattgttccacaaagtttccttaaagacgattcaatagacaataaggtcttaacgcgttctgataaaaatcgtggtaaatcggataacgttccaagtgaagaagtagtcaaaaagatgaaaaactattggagacaacttctaaacgccaagttaatcactcaacgtaagtttgataatttaacgaaagctgaacgtggaggtttgagtgaacttgataaagctggttttatcaaacgccaattggttgaaactcgccaaatcactaagcatgtggcacaaattttggatagtcgcatgaatactaaatacgatgaaaatgataaacttattcgagaggttaaagtgattaccttaaaatctaaattagtttctgacttccgaaaagatttccaattctataaagtacgtgagattaacaattaccatcatgcccatgatgcgtatctaaatgccgtcgttggaactgctttgattaagaaatatccaaaacttgaatcggagtttgtctatggtgattataaagtttatgatgttcgtaaaatgattgctaagtctgagcaagaaataggcaaagcaaccgcaaaatatttcttttactctaatatcatgaacttcttcaaaacagaaattacacttgcaaatggagagattcgcaaacgccctctaatcgaaactaatggggaaactggagaaattgtctgggataaagggcgagattttgccacagtgcgcaaagtattgtccatgccccaagtcaatattgtcaagaaaacagaagtacagacaggcggattctccaaggagtcaattttaccaaaaagaaattcggacaagcttattgctcgtaaaaaagactgggatccaaaaaaatatggtggttttgatagtccaacggtagcttattcagtcctagtggttgctaaggtggaaaaagggaaatcgaagaagttaaaatccgttaaagagttactagggatcacaattatggaaagaagttcctttgaaaaaaatccgattgactttttagaagctaaaggatataaggaagttaaaaaagacttaatcattaaactacctaaatatagtctttttgagttagaaaacggtcgtaaacggatgctggctagtgccggagaattacaaaaaggaaatgagctggctctgccaagcaaatatgtgaattttttatatttagctagtcattatgaaaagttgaagggtagtccagaagataacgaacaaaaacaattgtttgtggagcagcataagcattatttagatgagattattgagcaaatcagtgaattttctaagcgtgttattttagcagatgccaatttagataaagttcttagtgcatataacaaacatagagacaaaccaatacgtgaacaagcagaaaatattattcatttatttacgttgacgaatcttggagctcccgctgcttttaaatattttgatacaacaattgatcgtaaacgatatacgtctacaaaagaagttttagatgccactcttatccatcaatccatcactggtctttatgaaacacgcattgatttgagtcagctaggaggtgactaacgcatcctcacgataatatccgggtaggcgcaatcactttcgtctactccgttacaaagcgaggctgggtatttcccggcctttctgttatccgaaatccactgaaagcacagcggctggctgaggagataaataataaacgaggggctgtatgcacaaagcatcttctgttgagttaagaacgagtatcgagatggcacatagccttgctcaaattggaatcaggtttgtgccaataccagtagaaacagacgaagaatccatgggtatggacagttttccctttgatatgtaacggtgaacagttgttctacttttgtttgttagtcttgatgcttcactgatagatacaagagccaaatctagtaatattttatctgattaataagatgatcttcttgagatcgttttggtctgcgcgtaatctcttgctctgaaaacgaaaaaaccgccttgcagggcggtttttcgaaggttctctgagctaccaactctttgaaccgaggtaactggcttggaggagcgcagtcaccaaaacttgtcctttcagtttagccttaaccggcgcatgacttcaagactaactcctctaaatcaattaccagtggctgctgccagtggtgcttttgcatgtctttccgggttggactcaagacgatagttaccggataaggcgcagcggtcggactgaacggggggttcgtgcatacagtccagcttggagcgaactgcctacccggaactgagtgtcaggcgtggaatgagacaaacgcggccataacagcggaatgacaccggtaaaccgaaaggcaggaacaggagagcgcacgagggagccgccagggggaaacgcctggtatctttatagtcctgtcgggtttcgccaccactgatttgagcgtcagatttcgtgatgcttgtcaggggggcggagcctatggaaaaacggctttgccgcggccccgctgaatattccttttgtctccgaccatcaggcacctgagtcgctgtctttttcgtgacattcagttcgctgcgctcacggctctggcagtgaatgggggtaaatggcactacaggcgccttttatggattcatgcaaggaaactacccataatacaagaaaagatgtggtctttattcttcaactaaagcacccattagttcaacaaacgaaaattggataaagtgggatatttttaaaatatatatttatgttacctggcagagcctgtactttttacagtcggttttctaatgtcactaacctgccccgttagtcgccatttgcatcgatttattatgacaacttgacggctacatcattcactttttcttcacaaccggcacggaactcgctcgggctggccccggtgcattttttaaatacccgcgagaaatagagttgatcgtcaaaaccaacattgcgaccgacggtggcgataggcatccgggtggtgctcaaaagcagcttcgcctggctgatacgttggtcctcgcgccagcttaagacgctaatccctaactgctggcggaaaagatgtgacagacgcgacggcgacaagcaaacatgctgtgcgacgctggcgatatcaaaattgctgtctgccaggtgatcgctgatgtactgacaagcctcgcgtacccgattatccatcggtggatggagcgactcgttaatcgcttccatgcgccgcagtaacaattgctcaagcagatttatcgccagcagctccgaatagcgcccttccccttgcccggcgttaatgatttgcccaaacaggtcgctgaaatgcggctggtgcgcttcatccgggcgaaagaaccccgtattggcaaatattgacggccagttaagccattcatgccagtaggcgcgcggacgaaagtaaacccactggtgataccattcgcgagcctccggatgacgaccgtagtgatgaatctctcctggcgggaacagcaaaatatcacccggtcggcaaacaaattctcgtccctgatttttcaccaccccctgaccgcgaatggtgagattgagaatataacctttcattcccagcggtcggtcgataaaaaaatcgagataaccgttggcctcaatcggcgttaaacccgccaccagatgggcattaaacgagtatcccggcagcaggggatcattttgcgcttcagccatacttttcatactcccgccattcagagaagaaaccaattgtccatattgcatcagacattgccgtcactgcgtcttttactggctcttctcgctaaccaaaccggtaaccccgcttattaaaagcattctgtaacaaagcgggaccagtaatagaaagtgagggagccacggttgatgagagctttgttgtaggtggaccagttggtgattttgaacttttgctttgccacggaacggtctgcgttgtcgggaagatgcgtgatctgatccttcaactcagcaaaagttcgatttattcaacaaagccacgttgtgtctcaaaatctctgatgttacattgcacaagataaaaatatatcatcatgaacaataaaactgtctgcttacataaacagtaatacaaggggtgttatgagccatattcaacgggaaacgtcttgctcgaggccgcgattaaattccaacatggatgctgatttatatgggtataaatgggctcgcgataatgtcgggcaatcaggtgcgacaatctatcgattgtatgggaagcccgatgcgccagagttgtttctgaaacatggcaaaggtagcgttgccaatgatgttacagatgagatggtcagactaaactggctgacggaatttatgcctcttccgaccatcaagcattttatccgtactcctgatgatgcatggttactcaccactgcgatccccgggaaaacagcattccaggtattagaagaatatcctgattcaggtgaaaatattgttgatgcgctggcagtgttcctgcgccggttgcattcgattcctgtttgtaattgtccttttaacagcgatcgcgtatttcgtctcgctcaggcgcaatcacgaatgaataacggtttggttgatgcgagtgattttgatgacgagcgtaatggctggcctgttgaacaagtctggaaagaaatgcataagcttttgccattctcaccggattcagtcgtcactcatggtgatttctcacttgataaccttatttttgacgaggggaaattaataggttgtattgatgttggacgagtcggaatcgcagaccgataccaggatcttgccatcctatggaactgcctcggtgagttttctccttcattacagaaacggctttttcaaaaatatggtattgataatcctgatatgaataaattgcagtttcatttgatgctcgatgagtttttctaatcagaattggttaattggttgtaaca